European Patent Application EP 4 349 865 A1, published April 10, 2024. Title: PHARMACEUTICAL COMPOSITION CONTAINING ANTIBODY SPECIFICALLY BINDING TO ASM PROTEIN AS ACTIVE INGREDIENT FOR TREATING BRAIN DISEASE. Applicant: ISU ABXIS CO., LTD. KYUNGBOOK NATIONAL UNIVERSITY INDUSTRY-ACADEMIC COOPERATION FOUNDATION. The sequence listing filed with the application follows.

SEQUENCE LISTING (77 sequences)

SEQ ID NO: 1 - protein, 116 aa, Artificial Sequence
  #9101 heavy chain variable region amino acid sequence
EVQLLESGGGLVQPGGSLRLSCAASGFTFSNYAMSWVRQAPGKGLEWVSGIYPNGGNKYYADSVKGRFTISRDNSKNTLYLQMNSLRAEDTAVYYCAKNAYRFDYWGQGTLVTVSS

SEQ ID NO: 2 - DNA, 348 bp, Artificial Sequence
  #9101 heavy chain variable region nucleotide sequence
gaggtgcagctgttggagtctgggggaggcttggtacagcctggggggtccctgagactctcctgtgcagcctccggattcacctttagcaattatgctatgagctgggtccgccaggctccagggaaggggctggagtgggtctcagggatctatcctaatggtggtaataaatattacgctgattctgtaaaaggtcggttcaccatctccagagacaattccaagaacacgctgtatctgcaaatgaacagcctgagagccgaggacacggccgtgtattactgtgcgaaaaatgcttatcgtttcgactactggggccagggtacactggtcaccgtgagctca

SEQ ID NO: 3 - protein, 116 aa, Artificial Sequence
  #9102 heavy chain variable region amino acid sequence
EVQLLESGGGLVQPGGSLRLSCAASGFTFSGYYMSWVRQAPGKGLEWVSLISPGSGSIYYADSVKGRFTISRDNSKNTLYLQMNSLRAEDTAVYYCAKSWHHFDYWGQGTLVTVSS

SEQ ID NO: 4 - DNA, 348 bp, Artificial Sequence
  #9102 heavy chain variable region nucleotide sequence
gaggtgcagctgttggagtctgggggaggcttggtacagcctggggggtccctgagactctcctgtgcagcctccggattcacctttagcggttattatatgagctgggtccgccaggctccagggaaggggctggagtgggtctcattgatctctcctggtagtggtagtatatattacgctgattctgtaaaaggtcggttcaccatctccagagacaattccaagaacacgctgtatctgcaaatgaacagcctgagagccgaggacacggccgtgtattactgtgcgaaatcttggcatcatttcgactactggggccagggtacactggtcaccgtgagctca

SEQ ID NO: 5 - protein, 116 aa, Artificial Sequence
  #9104 heavy chain variable region amino acid sequence
EVQLLESGGGLVQPGGSLRLSCAASGFTFSNYYMSWVRQAPGKGLEWVSGIYYGSGNIYYADSVKGRFTISRDNSKNTLYLQMNSLRAEDTAVYYCARDTPGFDYWGQGTLVTVSS

SEQ ID NO: 6 - DNA, 348 bp, Artificial Sequence
  #9104 heavy chain variable region nucleotide sequence
gaggtgcagctgttggagtctgggggaggcttggtacagcctggggggtccctgagactctcctgtgcagcctccggattcacctttagcaattattatatgagctgggtccgccaggctccagggaaggggctggagtgggtctcagggatctattatggtagtggtaatatatattacgctgattctgtaaaaggtcggttcaccatctccagagacaattccaagaacacgctgtatctgcaaatgaacagcctgagagccgaggacacggccgtgtattactgtgcgagagatacgcctgggttcgactactggggccagggtacactggtcaccgtgagctca

SEQ ID NO: 7 - protein, 121 aa, Artificial Sequence
  #9108 heavy chain variable region amino acid sequence
EVQLLESGGGLVQPGGSLRLSCAASGFTFSNYAMSWVRQAPGKGLEWVSAIYPGGGSIYYADSVKGRFTISRDNSKNTLYLQMNSLRAEDTAVYYCARDVLGLTPKPFDYWGQGTLVTVSS

SEQ ID NO: 8 - DNA, 363 bp, Artificial Sequence
  #9108 heavy chain variable region nucleotide sequence
gaggtgcagctgttggagtctgggggaggcttggtacagcctggggggtccctgagactctcctgtgcagcctccggattcacctttagcaattatgctatgagctgggtccgccaggctccagggaaggggctggagtgggtctcagcgatctatcctggtggtggtagtatatattacgctgattctgtaaaaggtcggttcaccatctccagagacaattccaagaacacgctgtatctgcaaatgaacagcctgagagccgaggacacggccgtgtattactgtgcgagagatgttttgggtctgactcctaagccgttcgactactggggccagggtacactggtcaccgtgagctca

SEQ ID NO: 9 - protein, 116 aa, Artificial Sequence
  #9113 heavy chain variable region amino acid sequence
EVQLLESGGGLVQPGGSLRLSCAASGFTFSSYYMSWVRQAPGKGLEWVSSISPGGSSIYYADSVKGRFTISRDNSKNTLYLQMNSLRAEDTAVYYCAKGASLFDYWGQGTLVTVSS

SEQ ID NO: 10 - DNA, 348 bp, Artificial Sequence
  #9113 heavy chain variable region nucleotide sequence
gaggtgcagctgttggagtctgggggaggcttggtacagcctggggggtccctgagactctcctgtgcagcctccggattcacctttagcagttattatatgagctgggtccgccaggctccagggaaggggctggagtgggtctcatcgatctctcctggtggtagtagtatatattacgctgattctgtaaaaggtcggttcaccatctccagagacaattccaagaacacgctgtatctgcaaatgaacagcctgagagccgaggacacggccgtgtattactgtgcgaaaggggcgtctctgttcgactactggggccagggtacactggtcaccgtgagctca

SEQ ID NO: 11 - protein, 127 aa, Artificial Sequence
  #9123 heavy chain variable region amino acid sequence
EVQLLESGGGLVQPGGSLRLSCAASGFTFSDYAMSWVRQAPGKGLEWVSAISYGGGNIYYADSVKGRFTISRDNSKNTLYLQMNSLRAEDTAVYYCARVGGMCTRRQCYYDYGMDVWGQGTLVTVSS

SEQ ID NO: 12 - DNA, 381 bp, Artificial Sequence
  #9123 heavy chain variable region nucleotide sequence
gaggtgcagctgttggagtctgggggaggcttggtacagcctggggggtccctgagactctcctgtgcagcctccggattcacctttagcgattatgctatgagctgggtccgccaggctccagggaaggggctggagtgggtctcagcgatctcttatggtggtggtaatatatattacgctgattctgtaaaaggtcggttcaccatctccagagacaattccaagaacacgctgtatctgcaaatgaacagcctgagagccgaggacacggccgtgtattactgtgcgagagttggtggtatgtgtactaggcgtcagtgttattatgattatggtatggacgtctggggccagggtacactggtcaccgtgagctca

SEQ ID NO: 13 - protein, 110 aa, Artificial Sequence
  #9101 light chain variable region amino acid sequence
QSVLTQPPSASGTPGQRVTISCSGSSSNIGNNYVSWYQQLPGTAPKLLIYADSKRPSGVPDRFSGSKSGTSASLAIGGLRSEDEADYYCGSWDYSLNAYVFGGGTKLTVL

SEQ ID NO: 14 - DNA, 330 bp, Artificial Sequence
  #9101 light chain variable region nucleotide sequence
cagtctgtgctgactcagccaccctcagctagcgggacccccgggcagagggtcaccatctcttgtagtggctcttcatccaatattggcaataattatgtctcctggtaccagcagctcccaggaacggcccccaaactcctcatctatgctgatagtaagcggccaagcggggtccctgaccgattctctggctccaagtctggcacctcagcctcgctggccatcggtgggctccggtccgaggatgaggctgattattactgtggttcttgggattatagcctgaatgcttatgtcttcggcggaggcaccaagcttacggtccta

SEQ ID NO: 15 - protein, 110 aa, Artificial Sequence
  #9102 light chain variable region amino acid sequence
QSVLTQPPSASGTPGQRVTISCSGSSSNIGNNPVYWYQQLPGTAPKLLIYANNQRPSGVPDRFSGSKSGTSASLAISGLRSEDEADYYCAAWDSSLSGYVFGGGTKLTVL

SEQ ID NO: 16 - DNA, 330 bp, Artificial Sequence
  #9102 light chain variable region nucleotide sequence
cagtctgtgctgactcagccaccctcagctagcgggacccccgggcagagggtcaccatctcttgtagtggctcttcatctaatattggcaataatcctgtctactggtaccagcagctcccaggaacggcccccaaactcctcatctatgctaataatcagcggccaagcggggtccctgaccgattctctggctccaagtctggcacctcagcctccctggccatcagtgggctccggtccgaggatgaggctgattattactgtgctgcttgggattctagcctgagtggttatgtcttcggcggaggcaccaagcttacggtccta

SEQ ID NO: 17 - protein, 110 aa, Artificial Sequence
  #9104 light chain variable region amino acid sequence
QSVLTQPPSASGTPGQRVTISCTGSSSNIGNNAVNWYQQLPGTAPKLLIYYDSHRPSGVPDRFSGSKSGTSASLAISGLRSEDEADYYCGAWDYSLSAYVFGGGTKLTVL

SEQ ID NO: 18 - DNA, 330 bp, Artificial Sequence
  #9104 light chain variable region nucleotide sequence
cagtctgtgctgactcagccaccctcagctagcgggacccccgggcagagggtcaccatctcttgtactggctcttcatctaatattggcaataatgctgtcaactggtaccagcagctcccaggaacggcccccaaactcctcatctattatgatagtcatcggccaagcggggtccctgaccgattctctggctccaagtctggcacctcagcctccctggccatcagtgggctccggtccgaggatgaggctgattattactgtggtgcttgggattatagcctgagtgcttatgtcttcggcggaggcaccaagcttacggtccta

SEQ ID NO: 19 - protein, 110 aa, Artificial Sequence
  #9108 light chain variable region amino acid sequence
QSVLTQPPSASGTPGQRVTLSCTGSSSNIGSNTVYWYQQLPGTAPKLLIYANSQRPSGVPDRFSGSKSGTSASLAISGLRSEDEADYYCGSWDYSLSGYVFGGGTKLTVL

SEQ ID NO: 20 - DNA, 330 bp, Artificial Sequence
  #9108 light chain variable region nucleotide sequence
cagtctgtgctgactcagccaccctcagctagcgggacccccgggcagagggtcaccctctcttgtactggctcttcatctaatattggcagtaatactgtctactggtaccagcagctcccaggaacggcccccaaactcctcatctatgctaatagtcagcggccaagcggggtccctgaccgattctctggctccaagtctggcacctcagcctccctggccatcagtgggctccggtccgaggatgaggctgattattactgtggttcttgggattatagcctgagtggttatgtcttcggcggaggcaccaagcttacggtccta

SEQ ID NO: 21 - protein, 110 aa, Artificial Sequence
  #9113 light chain variable region amino acid sequence
QSVLTQPPSASGTPGQRVTISCSGSSSNIGNNAVSWYQQLPGTAPKLLIYSDNKRPSGVPDRFSGSKSGTSASLAISGLRSEDEADYYCGTWDASLNAYVFGGGTKLTVL

SEQ ID NO: 22 - DNA, 330 bp, Artificial Sequence
  #9113 light chain variable region nucleotide sequence
cagtctgtgctgactcagccaccctcagctagtgggacccccgggcagagggtcaccatctcttgtagtggctcttcatctaatattggcaataatgctgtctcctggtaccagcagctcccaggaacggcccccaaactcctcatctattctgataataagcggccaagcggggtccctgaccgattctctggctccaagtctggcacctcagcctccctggccatcagtgggctccggtccgaggatgaggctgattattactgtggtacttgggatgctagcctgaatgcttatgtcttcggcggaggcaccaagcttacggtccta

SEQ ID NO: 23 - protein, 110 aa, Artificial Sequence
  #9123 light chain variable region amino acid sequence
QSVLTQPPSASGTPGQRVTISCSGSSSNIGSNTVNWYQQLPGTAPKLLIYDNSKRPSGVPDRFSGSKSGTSASLAISGLRSEDEADYYCGTWDDSLSGYVFGGGTKLTVL

SEQ ID NO: 24 - DNA, 330 bp, Artificial Sequence
  #9123 light chain variable region nucleotide sequence
cagtctgtgctgactcagccaccctcagctagcgggacccccgggcagagggtcaccatctcttgtagtggctcttcatctaatattggcagtaatactgtcaactggtaccagcagctcccaggaacggcccccaaactcctcatctatgataatagtaagcggccaagcggggtccctgaccgattctctggctccaagtctggcacctcagcctccctggccatcagtgggctccggtccgaagatgaggctgattattactgtggtacttgggatgatagcctgagtggttatgtcttcggcggaggcaccaagcttacggtccta

SEQ ID NO: 25 - protein, 5 aa, Artificial Sequence
  #9101 heavy chain CDR1
NYAMS

SEQ ID NO: 26 - protein, 17 aa, Artificial Sequence
  #9101 heavy chain CDR2
GIYPNGGNKYYADSVKG

SEQ ID NO: 27 - protein, 7 aa, Artificial Sequence
  #9101 heavy chain CDR3
NAYRFDY

SEQ ID NO: 28 - protein, 5 aa, Artificial Sequence
  #9102 heavy chain CDR1
GYYMS

SEQ ID NO: 29 - protein, 17 aa, Artificial Sequence
  #9102 heavy chain CDR2
LISPGSGSIYYADSVKG

SEQ ID NO: 30 - protein, 7 aa, Artificial Sequence
  #9102 heavy chain CDR3
SWHHFDY

SEQ ID NO: 31 - protein, 5 aa, Artificial Sequence
  #9104 heavy chain CDR1
NYYMS

SEQ ID NO: 32 - protein, 17 aa, Artificial Sequence
  #9104 heavy chain CDR2
GIYYGSGNIYYADSVKG

SEQ ID NO: 33 - protein, 7 aa, Artificial Sequence
  #9104 heavy chain CDR3
DTPGFDY

SEQ ID NO: 34 - protein, 5 aa, Artificial Sequence
  #9108 heavy chain CDR1
NYAMS

SEQ ID NO: 35 - protein, 17 aa, Artificial Sequence
  #9108 heavy chain CDR2
AIYPGGGSIYYADSVKG

SEQ ID NO: 36 - protein, 12 aa, Artificial Sequence
  #9108 heavy chain CDR3
DVLGLTPKPFDY

SEQ ID NO: 37 - protein, 5 aa, Artificial Sequence
  #9113 heavy chain CDR1
SYYMS

SEQ ID NO: 38 - protein, 17 aa, Artificial Sequence
  #9113 heavy chain CDR2
SISPGGSSIYYADSVKG

SEQ ID NO: 39 - protein, 7 aa, Artificial Sequence
  #9113 heavy chain CDR3
GASLFDY

SEQ ID NO: 40 - protein, 5 aa, Artificial Sequence
  #9123 heavy chain CDR1
DYAMS

SEQ ID NO: 41 - protein, 17 aa, Artificial Sequence
  #9123 heavy chain CDR2
AISYGGGNIYYADSVKG

SEQ ID NO: 42 - protein, 18 aa, Artificial Sequence
  #9123 heavy chain CDR3
VGGMCTRRQCYYDYGMDV

SEQ ID NO: 43 - protein, 13 aa, Artificial Sequence
  #9101 light chain CDR1
SGSSSNIGNNYVS

SEQ ID NO: 44 - protein, 7 aa, Artificial Sequence
  #9101 light chain CDR2
ADSKRPS

SEQ ID NO: 45 - protein, 11 aa, Artificial Sequence
  #9101 light chain CDR3
GSWDYSLNAYV

SEQ ID NO: 46 - protein, 13 aa, Artificial Sequence
  #9102 light chain CDR1
SGSSSNIGNNPVY

SEQ ID NO: 47 - protein, 7 aa, Artificial Sequence
  #9102 light chain CDR2
ANNQRPS

SEQ ID NO: 48 - protein, 11 aa, Artificial Sequence
  #9102 light chain CDR3
AAWDSSLSGYV

SEQ ID NO: 49 - protein, 13 aa, Artificial Sequence
  #9104 light chain CDR1
TGSSSNIGNNAVN

SEQ ID NO: 50 - protein, 7 aa, Artificial Sequence
  #9104 light chain CDR2
YDSHRPS

SEQ ID NO: 51 - protein, 11 aa, Artificial Sequence
  #9104 light chain CDR3
GAWDYSLSAYV

SEQ ID NO: 52 - protein, 13 aa, Artificial Sequence
  #9108 light chain CDR1
TGSSSNIGSNTVY

SEQ ID NO: 53 - protein, 7 aa, Artificial Sequence
  #9108 light chain CDR2
ANSQRPS

SEQ ID NO: 54 - protein, 11 aa, Artificial Sequence
  #9108 light chain CDR3
GSWDYSLSGYV

SEQ ID NO: 55 - protein, 13 aa, Artificial Sequence
  #9113 light chain CDR1
SGSSSNIGNNAVS

SEQ ID NO: 56 - protein, 7 aa, Artificial Sequence
  #9113 light chain CDR2
SDNKRPS

SEQ ID NO: 57 - protein, 11 aa, Artificial Sequence
  #9113 light chain CDR3
GTWDASLNAYV

SEQ ID NO: 58 - protein, 13 aa, Artificial Sequence
  #9123 light chain CDR1
SGSSSNIGSNTVN

SEQ ID NO: 59 - protein, 7 aa, Artificial Sequence
  #9123 light chain CDR2
DNSKRPS

SEQ ID NO: 60 - protein, 11 aa, Artificial Sequence
  #9123 light chain CDR3
GTWDDSLSGYV

SEQ ID NO: 61 - protein, 5 aa, Artificial Sequence
  heavy chain CDR1
XYXMS

SEQ ID NO: 62 - protein, 17 aa, Artificial Sequence
  heavy chain CDR2
XIXXXXXXXYYADSVKG

SEQ ID NO: 63 - protein, 13 aa, Artificial Sequence
  light chain CDR1
XGSSSNIGXNXVX

SEQ ID NO: 64 - protein, 7 aa, Artificial Sequence
  light chain CDR2
XXXXRPS

SEQ ID NO: 65 - protein, 11 aa, Artificial Sequence
  light chain CDR3
XXWDXSLXXYV

SEQ ID NO: 66 - protein, 584 aa, Artificial Sequence
  human ASM protein
LALSDSRVLWAPAEAHPLSPQGHPARLHRIVPRLRDVFGWGNLTCPICKGLFTAINLGLKKEPNVARVGSVAIKLCNLLKIAPPAVCQSIVHLFEDDMVEVWRRSVLSPSEACGLLLGSTCGHWDIFSSWNISLPTVPKPPPKPPSPPAPGAPVSRILFLTDLHWDHDYLEGTDPDCADPLCCRRGSGLPPASRPGAGYWGEYSKCDLPLRTLESLLSGLGPAGPFDMVYWTGDIPAHDVWHQTRQDQLRALTTVTALVRKFLGPVPVYPAVGNHESTPVNSFPPPFIEGNHSSRWLYEAMAKAWEPWLPAEALRTLRIGGFYALSPYPGLRLISLNMNFCSRENFWLLINSTDPAGQLQWLVGELQAAEDRGDKVHIIGHIPPGHCLKSWSWNYYRIVARYENTLAAQFFGHTHVDEFEVFYDEETLSRPLAVAFLAPSATTYIGLNPGYRVYQIDGNYSGSSHVVLDHETYILNLTQANIPGAIPHWQLLYRARETYGLPNTLPTAWHNLVYRMRGDMQLFQTFWFLYHKGHPPSEPCGTPCRLATLCAQLSARADSPALCRHLMPDGSLPEAQSLWPRPLF

SEQ ID NO: 67 - protein, 582 aa, Artificial Sequence
  mouse ASM protein
LFDSTVLWVPARAYPLPSEGHSVKFSAIAPPLQSAFGWQNLTCPACKVLFTALNHGLKKEPNVARVGSVAIKICKMLNIAPLDVCQSAVHLFEDDVVEVWTRSVLSPSEACGLLLGSSCGHWDIFSTWNISLPSVPKPPPKPPSPPAPGAPVSRVLFLTDLHWDHEYLEGTDPYCADPLCCRRGSGWPPNSQKGAGFWGEYSKCDLPLRTLESLLKGLGPAGPFEMVYWTGDIPAHDVWQQSRQDQLRALTTITDLVRKFLGPVPVYPAVGNHESTPVNGFPPPFIKGNQSSQWLYEAMAKAWEPWLPADALHTLRIGGFYALTPRPGLRLISLNMNFCSRENFWLLINSTDPAGQLQWLVEELQAAENRGDKVHIIGHIPPGHCLKSWSWNYYKIIARYENTLAGQFFGHTHVDEFEIFYDEETLSRPLAVAFLAPSATTFINLNPGYRVYQIDGNYPGSSHVVLDHETYILNLTQANAAGGTPSWKRLYRARETYGLPDAMPASWHNLVYRMRDDEQLFQTFWFLYHKGHPPSEPCGTPCRLATLCAQLSARADSPALCRHLMPNGSLPDANRLWSRPLL

SEQ ID NO: 68 - protein, 20 aa, Artificial Sequence
  epitope of ASM protein (53-72)
TAINLGLKKEPNVARVGSVA

SEQ ID NO: 69 - protein, 23 aa, Artificial Sequence
  epitope of ASM protein (101-123)
VWRRSVLSPSEACGLLLGSTCGH

SEQ ID NO: 70 - protein, 25 aa, Artificial Sequence
  epitope of ASM protein (135-159)
PTVPKPPPKPPSPPAPGAPVSRILF

SEQ ID NO: 71 - protein, 21 aa, Artificial Sequence
  epitope of ASM protein (135-155)
PTVPKPPPKPPSPPAPGAPVS

SEQ ID NO: 72 - protein, 11 aa, Artificial Sequence
  epitope of ASM protein (218-228)
SGLGPAGPFDM

SEQ ID NO: 73 - protein, 11 aa, Artificial Sequence
  epitope of ASM protein (259-269)
VRKFLGPVPVY

SEQ ID NO: 74 - protein, 324 aa, Artificial Sequence
  Mouse IgG1 heavy chain constant region amino acid sequence
AKTTPPSVYPLAPGSAAQTNSMVTLGCLVKGYFPEPVTVTWNSGSLSSGVHTFPAVLQSDLYTLSSSVTVPSSPRPSETVTCNVAHPASSTKVDKKIVPRDCGCKPCICTVPEVSSVFIFPPKPKDVLTITLTPKVTCVVVDISKDDPEVQFSWFVDDVEVHTAQTQPREEQFNSTFRSVSELPIMHQDWLNGKEFKCRVNSAAFPAPIEKTISKTKGRPKAPQVYTIPPPKEQMAKDKVSLTCMITDFFPEDITVEWQWNGQPAENYKNTQPIMNTNGSYFVYSKLNVQKSNWEAGNTFTCSVLHEGLHNHHTEKSLSHSPGK

SEQ ID NO: 75 - DNA, 972 bp, Artificial Sequence
  Mouse IgG1 heavy chain constant region nucleotide sequence
gccaagacaacacctcctagcgtgtaccctctggctcctggatctgccgctcagaccaatagcatggtcaccctgggctgtctggtcaagggctactttcctgagcctgtgaccgtgacctggaacagcggatctctgtctagcggcgtgcacacctttccagccgtgctgcagagcgatctgtacaccctgagcagcagcgtgaccgtgcctagctctcctagacctagcgagacagtgacctgcaacgtggcccatcctgccagcagcaccaaggtggacaagaaaatcgtgcccagagactgcggctgcaagccctgcatctgtaccgtgcctgaagtgtccagcgtgttcatcttcccacctaagcctaaggacgtgctgaccatcacactgacccctaaagtgacctgtgtggtggtggacatcagcaaggacgaccccgaggtgcagttcagttggttcgtggacgacgtggaagtgcacacagcccagacacagcctagagaggaacagttcaacagcaccttcagaagcgtgtccgagctgcccatcatgcaccaggattggctgaacggcaaagaattcaagtgcagagtgaacagcgccgcctttcctgctcctatcgagaaaaccatctccaagaccaagggcagacccaaggctccccaggtgtacacaatccctccacctaaagaacagatggccaaggacaaggtgtccctgacctgcatgatcaccgatttcttcccagaggacatcaccgtggaatggcagtggaatggacagcccgccgagaactacaagaatacccagcctatcatgaacaccaacggcagctacttcgtgtacagcaagctgaacgtgcagaagtccaactgggaggccggcaacaccttcacctgttctgtgctgcacgagggcctgcacaatcaccacaccgagaagtccctgagccactctcctggcaag

SEQ ID NO: 76 - protein, 106 aa, Artificial Sequence
  Mouse light chain lambda constant region amino acid sequence
GQPKSSPSVTLFPPSSEELETNKATLVCTITDFYPGVVTVDWKVDGTPVTQGMETTQPSKQSNNKYMASSYLTLTARAWERHSSYSCQVTHEGHTVEKSLSRADCS

SEQ ID NO: 77 - DNA, 318 bp, Artificial Sequence
  Mouse light chain lambda constant region nucleotide sequence
ggccagcctaagagcagccctagcgtgaccctgtttcctccaagcagcgaggaactggaaacaaacaaggccacactcgtgtgcaccatcaccgacttctatcccggcgtggtcaccgtggattggaaggtggacggaacccctgtgacacaaggcatggaaaccacacagcccagcaagcagagcaacaacaagtacatggccagcagctacctgacactgaccgccagagcctgggagagacacagctcctacagctgccaagtgacacacgagggccacaccgtggaaaagtctctgagcagagccgactgcagc